European Patent Application EP 4 560 022 A2, published May 28, 2025. Title: LARGE GENE EXCISION AND INSERTION. Applicant: PRESIDENT AND FELLOWS OF HARVARD COLLEGE. Application WO PCT/US2014/066324, filed November 19, 2014. The sequence listing filed with the application follows.

SEQUENCE LISTING (120 sequences)

SEQ ID NO: 1 - protein, 1368 aa, Streptococcus pyogenes [sequence omitted]

SEQ ID NO: 2 - DNA, 22 bp, synthetic construct
  misc_feature 1..22: note = Target oligonucleotide
  source 1..22: mol_type = other DNA
cacagtctcagaaaagcgcagg

SEQ ID NO: 3 - DNA, 22 bp, synthetic construct
  misc_feature 1..22: note = Target oligonucleotide
  source 1..22: mol_type = other DNA
aaatatcagcgcggtggattgg

SEQ ID NO: 4 - DNA, 22 bp, synthetic construct
  misc_feature 1..22: note = Target oligonucleotide
  source 1..22: mol_type = other DNA
ggtcaggctgaactcgtactgg

SEQ ID NO: 5 - DNA, 22 bp, synthetic construct
  misc_feature 1..22: note = Target oligonucleotide
  source 1..22: mol_type = other DNA
ttagtagcaacgctaccccagg

SEQ ID NO: 6 - DNA, 22 bp, synthetic construct
  misc_feature 1..22: note = Target oligonucleotide
  source 1..22: mol_type = other DNA
gtgtgcagtcattagcccctgg

SEQ ID NO: 7 - DNA, 22 bp, synthetic construct
  misc_feature 1..22: note = Target oligonucleotide
  source 1..22: mol_type = other DNA
gggcaaatgtgtctcgttaggg

SEQ ID NO: 8 - DNA, 22 bp, synthetic construct
  misc_feature 1..22: note = Target oligonucleotide
  source 1..22: mol_type = other DNA
ttctcctttccgaagtccgtgg

SEQ ID NO: 9 - DNA, 22 bp, synthetic construct
  misc_feature 1..22: note = Target oligonucleotide
  source 1..22: mol_type = other DNA
gccgctgtcgcctggcaaaagg

SEQ ID NO: 10 - DNA, 22 bp, synthetic construct
  misc_feature 1..22: note = Target oligonucleotide
  source 1..22: mol_type = other DNA
gatggtagacatcgaccatggg

SEQ ID NO: 11 - DNA, 22 bp, synthetic construct
  misc_feature 1..22: note = Target oligonucleotide
  source 1..22: mol_type = other DNA
ttcaatttcgggcccgatctgg

SEQ ID NO: 12 - DNA, 22 bp, synthetic construct
  misc_feature 1..22: note = Target oligonucleotide
  source 1..22: mol_type = other DNA
tgagtcgcgtcacggctattgg

SEQ ID NO: 13 - DNA, 22 bp, synthetic construct
  misc_feature 1..22: note = Target oligonucleotide
  source 1..22: mol_type = other DNA
catttgcggtggtaatcgcagg

SEQ ID NO: 14 - DNA, 22 bp, synthetic construct
  misc_feature 1..22: note = Target oligonucleotide
  source 1..22: mol_type = other DNA
gatcggatcgggtcgcgtcggg

SEQ ID NO: 15 - DNA, 22 bp, synthetic construct
  misc_feature 1..22: note = Target oligonucleotide
  source 1..22: mol_type = other DNA
tttcctgcgctgaatcgggtgg

SEQ ID NO: 16 - DNA, 22 bp, synthetic construct
  misc_feature 1..22: note = Target oligonucleotide
  source 1..22: mol_type = other DNA
ggctcctgtctgtgcctgacgg

SEQ ID NO: 17 - DNA, 47 bp, synthetic construct
  misc_feature 1..47: note = PCR primer
  source 1..47: mol_type = other DNA
ctttcttgtacaaagttggcattattagacgtcaggtggcacttttc

SEQ ID NO: 18 - DNA, 47 bp, synthetic construct
  misc_feature 1..47: note = PCR primer
  source 1..47: mol_type = other DNA
cctttaaagcctgcttttttgtacagtttgcgtattgggcgctcttc

SEQ ID NO: 19 - DNA, 24 bp, synthetic construct
  misc_feature 1..24: note = PCR primer
  source 1..24: mol_type = other DNA
gccaccatggacaagaagtactcc

SEQ ID NO: 20 - DNA, 24 bp, synthetic construct
  misc_feature 1..24: note = PCR primer
  source 1..24: mol_type = other DNA
tcacaccttcctcttcttcttggg

SEQ ID NO: 21 - DNA, 48 bp, synthetic construct
  misc_feature 1..48: note = PCR primer
  source 1..48: mol_type = other DNA
ccgaaaagtgccacctgacgtcgacggatgaaaggagtgggaattggc

SEQ ID NO: 22 - DNA, 50 bp, synthetic construct
  misc_feature 1..50: note = PCR primer
  source 1..50: mol_type = other DNA
ggagtacttcttgtccatggtggcggccaactagccagcttgggtctccc

SEQ ID NO: 23 - DNA, 54 bp, synthetic construct
  misc_feature 1..54: note = PCR primer
  source 1..54: mol_type = other DNA
gctgaccccaagaagaagaggaaggtgtgacatcaccattgagtttaaacccgc

SEQ ID NO: 24 - DNA, 45 bp, synthetic construct
  misc_feature 1..45: note = PCR primer
  source 1..45: mol_type = other DNA
ccaagctctagctagaggtcgacggtatcgagccccagctggttc

SEQ ID NO: 25 - DNA, 21 bp, synthetic construct
  misc_feature 1..21: note = PCR primer
  source 1..21: mol_type = other DNA
ataccgtcgacctctagctag

SEQ ID NO: 26 - DNA, 18 bp, synthetic construct
  misc_feature 1..18: note = PCR primer
  source 1..18: mol_type = other DNA
tccgtcgacgtcaggtgg

SEQ ID NO: 27 - DNA, 23 bp, synthetic construct
  misc_feature 1..23: note = PCR primer
  source 1..23: mol_type = other DNA
tggtggtggttgtggtacacacc

SEQ ID NO: 28 - DNA, 21 bp, synthetic construct
  misc_feature 1..21: note = PCR primer
  source 1..21: mol_type = other DNA
aatagggagggccggggtacc

SEQ ID NO: 29 - DNA, 26 bp, synthetic construct
  misc_feature 1..26: note = PCR primer
  source 1..26: mol_type = other DNA
acccttcccctcctagatcccaagcc

SEQ ID NO: 30 - DNA, 52 bp, synthetic construct
  misc_feature 1..52: note = PCR primer
  source 1..52: mol_type = other DNA
gattaaaggtgtgtaccacaaccaccaccacttttctgagactgtgagggag

SEQ ID NO: 31 - DNA, 49 bp, synthetic construct
  misc_feature 1..49: note = PCR primer
  source 1..49: mol_type = other DNA
agactctggggtaccccggccctccctattcccaggggctaatgactgc

SEQ ID NO: 32 - DNA, 20 bp, synthetic construct
  misc_feature 1..20: note = PCR primer
  source 1..20: mol_type = other DNA
gcacctccagccatcacagc

SEQ ID NO: 33 - DNA, 53 bp, synthetic construct
  misc_feature 1..53: note = PCR primer
  source 1..53: mol_type = other DNA
ccaggaaggggctgtgatggctggaggtgcttagacgtcaggtggcacttttc

SEQ ID NO: 34 - DNA, 47 bp, synthetic construct
  misc_feature 1..47: note = PCR primer
  source 1..47: mol_type = other DNA
gggcttgggatctaggaggggaagggtttgcgtattgggcgctcttc

SEQ ID NO: 35 - DNA, 26 bp, synthetic construct
  misc_feature 1..26: note = PCR primer
  source 1..26: mol_type = other DNA
acccttcccctcctagatcccaagcc

SEQ ID NO: 36 - DNA, 20 bp, synthetic construct
  misc_feature 1..20: note = PCR primer
  source 1..20: mol_type = other DNA
gcacctccagccatcacagc

SEQ ID NO: 37 - DNA, 26 bp, synthetic construct
  misc_feature 1..26: note = PCR primer
  source 1..26: mol_type = other DNA
acccttcccctcctagatcccaagcc

SEQ ID NO: 38 - DNA, 33 bp, synthetic construct
  misc_feature 1..33: note = PCR primer
  source 1..33: mol_type = other DNA
aagattcagagagattcattcattcattcacaa

SEQ ID NO: 39 - DNA, 23 bp, synthetic construct
  misc_feature 1..23: note = PCR primer
  source 1..23: mol_type = other DNA
cctgctaacaggtacccggcatg

SEQ ID NO: 40 - DNA, 20 bp, synthetic construct
  misc_feature 1..20: note = PCR primer
  source 1..20: mol_type = other DNA
gcacctccagccatcacagc

SEQ ID NO: 41 - DNA, 25 bp, synthetic construct
  misc_feature 1..25: note = PCR primer
  source 1..25: mol_type = other DNA
cagcatcttgctaaggggttgtcag

SEQ ID NO: 42 - DNA, 25 bp, synthetic construct
  misc_feature 1..25: note = PCR primer
  source 1..25: mol_type = other DNA
gtcagcagacatgggatgttcgttt

SEQ ID NO: 43 - DNA, 47 bp, synthetic construct; identical to SEQ ID NO: 34
  misc_feature 1..47: note = PCR primer
  source 1..47: mol_type = other DNA

SEQ ID NO: 44 - DNA, 52 bp, synthetic construct
  misc_feature 1..52: note = PCR primer
  source 1..52: mol_type = other DNA
tgaatgaatgaatgaatctctctgaatcttgtttgcgtattgggcgctcttc

SEQ ID NO: 45 - DNA, 52 bp, synthetic construct
  misc_feature 1..52: note = PCR primer
  source 1..52: mol_type = other DNA
tcctgccccatgccgggtacctgttagcaggtttgcgtattgggcgctcttc

SEQ ID NO: 46 - DNA, 53 bp, synthetic construct; identical to SEQ ID NO: 33
  misc_feature 1..53: note = PCR primer
  source 1..53: mol_type = other DNA

SEQ ID NO: 47 - DNA, 53 bp, synthetic construct
  misc_feature 1..53: note = PCR primer
  source 1..53: mol_type = other DNA
ggaggctgacaaccccttagcaagatgctgttagacgtcaggtggcacttttc

SEQ ID NO: 48 - DNA, 53 bp, synthetic construct
  misc_feature 1..53: note = PCR primer
  source 1..53: mol_type = other DNA
caaataaacgaacatcccatgtctgctgacttagacgtcaggtggcacttttc

SEQ ID NO: 49 - DNA, 24 bp, synthetic construct
  misc_feature 1..24: note = PCR primer
  source 1..24: mol_type = other DNA
ccttcccctcctagatcccaagcc

SEQ ID NO: 50 - DNA, 20 bp, synthetic construct
  misc_feature 1..20: note = PCR primer
  source 1..20: mol_type = other DNA
gcacctccagccatcacagc

SEQ ID NO: 51 - DNA, 23 bp, synthetic construct
  misc_feature 1..23: note = PCR primer
  source 1..23: mol_type = other DNA
tcttgtttgagatgttgtgcggg

SEQ ID NO: 52 - DNA, 25 bp, synthetic construct
  misc_feature 1..25: note = PCR primer
  source 1..25: mol_type = other DNA
ctggtttcagcactccgatcctatc

SEQ ID NO: 53 - DNA, 20 bp, synthetic construct
  misc_feature 1..20: note = PCR primer
  source 1..20: mol_type = other DNA
tgtggctctgcaccaggaag

SEQ ID NO: 54 - DNA, 23 bp, synthetic construct
  misc_feature 1..23: note = PCR primer
  source 1..23: mol_type = other DNA
cctctcccttttccctggttttg

SEQ ID NO: 55 - DNA, 53 bp, synthetic construct
  misc_feature 1..53: note = PCR primer
  source 1..53: mol_type = other DNA
tactctgcaaaaccagggaaaagggagaggttagacgtcaggtggcacttttc

SEQ ID NO: 56 - DNA, 52 bp, synthetic construct
  misc_feature 1..52: note = PCR primer
  source 1..52: mol_type = other DNA
ctgtggataggatcggagtgctgaaaccaggtttgcgtattgggcgctcttc

SEQ ID NO: 57 - DNA, 54 bp, synthetic construct
  misc_feature 1..54: note = PCR primer
  source 1..54: mol_type = other DNA
atctctccacttcaggtgggtgggaggcccctgtggtctgtgtctccccaaatt

SEQ ID NO: 58 - DNA, 56 bp, synthetic construct
  misc_feature 1..56: note = PCR primer
  source 1..56: mol_type = other DNA
caggtggacaggaggacagattccagaggcttggttttattgtgcagttttctttc

SEQ ID NO: 59 - DNA, 19 bp, synthetic construct
  misc_feature 1..19: note = PCR primer
  source 1..19: mol_type = other DNA
ggcttccttccctccagag

SEQ ID NO: 60 - DNA, 17 bp, synthetic construct
  misc_feature 1..17: note = PCR primer
  source 1..17: mol_type = other DNA
acaggggcctcccaccc

SEQ ID NO: 61 - DNA, 22 bp, synthetic construct
  misc_feature 1..22: note = PCR primer
  source 1..22: mol_type = other DNA
caagcctctggaatctgtcctc

SEQ ID NO: 62 - DNA, 21 bp, synthetic construct
  misc_feature 1..21: note = PCR primer
  source 1..21: mol_type = other DNA
gcccagtgtgcagtcattagc

SEQ ID NO: 63 - DNA, 22 bp, synthetic construct
  misc_feature 1..22: note = PCR primer
  source 1..22: mol_type = other DNA
cttttctgagactgtgagggag

SEQ ID NO: 64 - DNA, 24 bp, synthetic construct
  misc_feature 1..24: note = PCR primer
  source 1..24: mol_type = other DNA
taccccaggggctaatgactgcac

SEQ ID NO: 65 - DNA, 28 bp, synthetic construct
  misc_feature 1..28: note = PCR primer
  source 1..28: mol_type = other DNA
acagtctcagaaaacgcaggtgacaaag

SEQ ID NO: 66 - DNA, 30 bp, synthetic construct
  misc_feature 1..30: note = PCR primer
  source 1..30: mol_type = other DNA
cattagcccctgggtagcgttgctactaag

SEQ ID NO: 67 - DNA, 29 bp, synthetic construct
  misc_feature 1..29: note = PCR primer
  source 1..29: mol_type = other DNA
ttgtcacctgcgttttctgagactgtgag

SEQ ID NO: 68 - DNA, 30 bp, synthetic construct
  misc_feature 1..30: note = PCR primer
  source 1..30: mol_type = other DNA
cttagtagcaacgctacccaggggctaatg

SEQ ID NO: 69 - DNA, 52 bp, synthetic construct
  misc_feature 1..52: note = PCR primer
  source 1..52: mol_type = other DNA
gagaataccagcagttcacccatccagtacgaaattctaccgggtaggggag

SEQ ID NO: 70 - DNA, 54 bp, synthetic construct
  misc_feature 1..54: note = PCR primer
  source 1..54: mol_type = other DNA
cccagtgtgcagtcattagcccctggggtacgacggccagtgaattgtaatacg

SEQ ID NO: 71 - DNA, 26 bp, synthetic construct
  misc_feature 1..26: note = PCR primer
  source 1..26: mol_type = other DNA
acccttcccctcctagatcccaagcc

SEQ ID NO: 72 - DNA, 28 bp, synthetic construct
  misc_feature 1..28: note = PCR primer
  source 1..28: mol_type = other DNA
gtactggatgggtgaactgctggtattc

SEQ ID NO: 73 - DNA, 24 bp, synthetic construct
  misc_feature 1..24: note = PCR primer
  source 1..24: mol_type = other DNA
taccccaggggctaatgactgcac

SEQ ID NO: 74 - DNA, 20 bp, synthetic construct
  misc_feature 1..20: note = PCR primer
  source 1..20: mol_type = other DNA
gcacctccagccatcacagc

SEQ ID NO: 75 - DNA, 53 bp, synthetic construct; identical to SEQ ID NO: 33
  misc_feature 1..53: note = PCR primer
  source 1..53: mol_type = other DNA

SEQ ID NO: 76 - DNA, 47 bp, synthetic construct; identical to SEQ ID NO: 34
  misc_feature 1..47: note = PCR primer
  source 1..47: mol_type = other DNA

SEQ ID NO: 77 - DNA, 69 bp, synthetic construct
  misc_feature 1..69: note = PCR primer
  source 1..69: mol_type = other DNA
gaagtcgaggttccaaggtcacagtgagggggccctggccaccccttgcaggttctccatagtccacag

SEQ ID NO: 78 - DNA, 25 bp, synthetic construct
  misc_feature 1..25: note = PCR primer
  source 1..25: mol_type = other DNA
caacaacccctcctgtatatgacct

SEQ ID NO: 79 - DNA, 25 bp, synthetic construct
  misc_feature 1..25: note = PCR primer
  source 1..25: mol_type = other DNA
acacactttcaacctccaagagacg

SEQ ID NO: 80 - DNA, 23 bp, synthetic construct
  misc_feature 1..23: note = PCR primer
  source 1..23: mol_type = other DNA
ctcactgtgaccttggaacctcg

SEQ ID NO: 81 - DNA, 51 bp, synthetic construct
  misc_feature 1..51: note = PCR primer
  source 1..51: mol_type = other DNA
tgttgaggtcatatacaggaggggttgttgcctgacggggttgggttttcc

SEQ ID NO: 82 - DNA, 23 bp, synthetic construct
  misc_feature 1..23: note = PCR primer
  source 1..23: mol_type = other DNA
aagggagccctgaggccttttcc

SEQ ID NO: 83 - DNA, 47 bp, synthetic construct
  misc_feature 1..47: note = PCR primer
  source 1..47: mol_type = other DNA
tcaggaaaaggcctcagggctcccttagacgtcaggtggcacttttc

SEQ ID NO: 84 - DNA, 47 bp, synthetic construct
  misc_feature 1..47: note = PCR primer
  source 1..47: mol_type = other DNA
cgtctcttggaggttgaaagtgtgtgtttgcgtattgggcgctcttc

SEQ ID NO: 85 - DNA, 18 bp, synthetic construct
  misc_feature 1..18: note = PCR primer
  source 1..18: mol_type = other DNA
taccagcagttcacccat

SEQ ID NO: 86 - DNA, 18 bp, synthetic construct
  misc_feature 1..18: note = PCR primer
  source 1..18: mol_type = other DNA
tctttgtctcacgggtca

SEQ ID NO: 87 - DNA, 18 bp, synthetic construct
  misc_feature 1..18: note = PCR primer
  source 1..18: mol_type = other DNA
tctccccaaccacttagt

SEQ ID NO: 88 - DNA, 18 bp, synthetic construct
  misc_feature 1..18: note = PCR primer
  source 1..18: mol_type = other DNA
tgtgcagtcattagcccc

SEQ ID NO: 89 - DNA, 25 bp, synthetic construct
  misc_feature 1..25: note = PCR primer
  source 1..25: mol_type = other DNA
ggccgccaccatggattataaggac

SEQ ID NO: 90 - DNA, 20 bp, synthetic construct
  misc_feature 1..20: note = PCR primer
  source 1..20: mol_type = other DNA
ggaacctgccactcgatgtg

SEQ ID NO: 91 - DNA, 44 bp, synthetic construct
  misc_feature 1..44: note = PCR primer
  source 1..44: mol_type = other DNA
gacatcacatcgagtggcaggttcccagctggtgaagtccgagc

SEQ ID NO: 92 - DNA, 63 bp, synthetic construct
  misc_feature 1..63: note = PCR primer
  source 1..63: mol_type = other DNA
caactagaaggcacagtcgaggctgatcagcggggttagaaattgatttcaccattgttgaac

SEQ ID NO: 93 - DNA, 50 bp, synthetic construct
  misc_feature 1..50: note = PCR primer
  source 1..50: mol_type = other DNA
gacatcacatcgagtggcaggttcccaactagtcaaaagtgaactggagg

SEQ ID NO: 94 - DNA, 54 bp, synthetic construct
  misc_feature 1..54: note = PCR primer
  source 1..54: mol_type = other DNA
caactagaaggcacagtcgaggctgatcagcgcccttaaaagtttatctcgccg

SEQ ID NO: 95 - DNA, 23 bp, synthetic construct
  misc_feature 1..23: note = PCR primer
  source 1..23: mol_type = other DNA
gcctcgactgtgccttctagttg

SEQ ID NO: 96 - DNA, 22 bp, synthetic construct
  misc_feature 1..22: note = PCR primer
  source 1..22: mol_type = other DNA
cttataatccatggtggcggcc

SEQ ID NO: 97 - DNA, 25 bp, synthetic construct
  misc_feature 1..25: note = PCR primer
  source 1..25: mol_type = other DNA
agggacttagatgactgccatagcc

SEQ ID NO: 98 - DNA, 25 bp, synthetic construct
  misc_feature 1..25: note = PCR primer
  source 1..25: mol_type = other DNA
atgttggcagtaagcatgttgttcc

SEQ ID NO: 99 - DNA, 25 bp, synthetic construct
  misc_feature 1..25: note = PCR primer
  source 1..25: mol_type = other DNA
agggacttagatgactgccatagcc

SEQ ID NO: 100 - DNA, 25 bp, synthetic construct
  misc_feature 1..25: note = PCR primer
  source 1..25: mol_type = other DNA
ctcacctctgagcactgtgacgttc

SEQ ID NO: 101 - DNA, 25 bp, synthetic construct
  misc_feature 1..25: note = PCR primer
  source 1..25: mol_type = other DNA
actgaagttctgggtcccaacaatg

SEQ ID NO: 102 - DNA, 25 bp, synthetic construct
  misc_feature 1..25: note = PCR primer
  source 1..25: mol_type = other DNA
atgaatacagactgcacctccccag

SEQ ID NO: 103 - DNA, 25 bp, synthetic construct
  misc_feature 1..25: note = PCR primer
  source 1..25: mol_type = other DNA
ctcacctctgagcactgtgacgttc

SEQ ID NO: 104 - DNA, 35 bp, synthetic construct
  misc_feature 1..35: note = PCR primer
  source 1..35: mol_type = other DNA
ccatcaatctactgaagttctgggtcccaacaatg

SEQ ID NO: 105 - DNA, 25 bp, synthetic construct
  misc_feature 1..25: note = PCR primer
  source 1..25: mol_type = other DNA
tgaagtgaaaccctaaagggggaag

SEQ ID NO: 106 - DNA, 25 bp, synthetic construct
  misc_feature 1..25: note = PCR primer
  source 1..25: mol_type = other DNA
aaaccacacacttcaacctggatgg

SEQ ID NO: 107 - DNA, 25 bp, synthetic construct
  misc_feature 1..25: note = PCR primer
  source 1..25: mol_type = other DNA
gtttggcccaagtttctaagggagg

SEQ ID NO: 108 - DNA, 70 bp, synthetic construct
  misc_feature 1..70: note = PCR primer
  source 1..70: mol_type = other DNA
tccctcacagtctcagaaaagcgcaggtgataaccacttagtagcaacgctaccccaggggctaatgact

SEQ ID NO: 109 - DNA, 38 bp, synthetic construct
  misc_feature 1..38: note = PCR primer
  source 1..38: mol_type = other DNA
tccctcacagtctcagaaaagcccaggggctaatgact

SEQ ID NO: 110 - DNA, 23 bp, synthetic construct
  misc_feature 1..23: note = PCR primer
  source 1..23: mol_type = other DNA
tccctcacagtctcagaatgact

SEQ ID NO: 111 - DNA, 38 bp, synthetic construct; identical to SEQ ID NO: 109
  misc_feature 1..38: note = PCR primer
  source 1..38: mol_type = other DNA

SEQ ID NO: 112 - DNA, 42 bp, synthetic construct
  misc_feature 1..42: note = PCR primer
  source 1..42: mol_type = other DNA
tccctcacagtctcagaactttatcaccaggggctaatgact

SEQ ID NO: 113 - DNA, 38 bp, synthetic construct; identical to SEQ ID NO: 109
  misc_feature 1..38: note = PCR primer
  source 1..38: mol_type = other DNA

SEQ ID NO: 114 - DNA, 59 bp, synthetic construct
  misc_feature 1..59: note = PCR primer
  source 1..59: mol_type = other DNA
tccctcacagtctcagaaaaggtagcgttgctatcacctgcgcccaggggctaatgact

SEQ ID NO: 115 - DNA, 39 bp, synthetic construct
  misc_feature 1..39: note = PCR primer
  source 1..39: mol_type = other DNA
tccctcacagtctcagaaaagccccaggggctaatgact

SEQ ID NO: 116 - DNA, 59 bp, synthetic construct; identical to SEQ ID NO: 114
  misc_feature 1..59: note = PCR primer
  source 1..59: mol_type = other DNA

SEQ ID NO: 117 - DNA, 39 bp, synthetic construct; identical to SEQ ID NO: 115
  misc_feature 1..39: note = PCR primer
  source 1..39: mol_type = other DNA

SEQ ID NO: 118 - DNA, 61 bp, synthetic construct
  misc_feature 1..61: note = PCR primer
  source 1..61: mol_type = other DNA
tccctcacagtctcagaaaagggtagcgttgctatcacctgcgccccaggggctaatgact

SEQ ID NO: 119 - DNA, 20 bp, synthetic construct
  misc_feature 1..20: note = PCR primer
  source 1..20: mol_type = other DNA
tccctcacagtctaatgact

SEQ ID NO: 120 - DNA, 59 bp, synthetic construct; identical to SEQ ID NO: 114
  misc_feature 1..59: note = PCR primer
  source 1..59: mol_type = other DNA